European Patent Application EP 4 789 668 A1, published August 12, 2026. Title: Atracurium salt for use in the treatment of bone fragility-related diseases. Applicant: Administracion General de la Comunidad Autonoma de Euskadi. The sequence listing filed with the application follows.

SEQUENCE LISTING (14 sequences)

SEQ ID NO: 1 - DNA, 20 bp, synthetic construct
  source 1..20: mol_type = other DNA
gggattccctggacctaaag

SEQ ID NO: 2 - DNA, 18 bp, synthetic construct
  source 1..18: mol_type = other DNA
ggaacacctcgctctcca

SEQ ID NO: 3 - DNA, 20 bp, synthetic construct
  source 1..20: mol_type = other DNA
agaggaccacgtggagaaag

SEQ ID NO: 4 - DNA, 18 bp, synthetic construct
  source 1..18: mol_type = other DNA
ggcctgtgggaccatctt

SEQ ID NO: 5 - DNA, 22 bp, synthetic construct
  source 1..22: mol_type = other DNA
acgagctgaacaggaacaacgt

SEQ ID NO: 6 - DNA, 22 bp, synthetic construct
  source 1..22: mol_type = other DNA
caccagcaagaagaagcctttg

SEQ ID NO: 7 - DNA, 22 bp, synthetic construct
  source 1..22: mol_type = other DNA
tggtgacagtgatcgtgctgca

SEQ ID NO: 8 - DNA, 22 bp, synthetic construct
  source 1..22: mol_type = other DNA
gcctcttcattcgcaggaacca

SEQ ID NO: 9 - DNA, 20 bp, synthetic construct
  source 1..20: mol_type = other DNA
caaggctgagaacgggaagc

SEQ ID NO: 10 - DNA, 20 bp, synthetic construct
  source 1..20: mol_type = other DNA
agggggcagagatgatgacc

SEQ ID NO: 11 - DNA, 28 bp, synthetic construct
  source 1..28: mol_type = other DNA
actgtctgtctacagtgaacgtcttaat

SEQ ID NO: 12 - DNA, 28 bp, synthetic construct
  source 1..28: mol_type = other DNA
gatgtagatgcatagaagacatggaagg

SEQ ID NO: 13 - DNA, 30 bp, synthetic construct
  source 1..30: mol_type = other DNA
ttcccatttttttctattatacagaaacag

SEQ ID NO: 14 - DNA, 28 bp, synthetic construct
  source 1..28: mol_type = other DNA
aatgattgtcttgccccattcatttttt